European Patent Specification EP 4 047 085 B1, published February 26, 2025. Title: NOVEL BRANCHED-CHAIN AMINO ACID AMINOTRANSFERASE VARIANT AND METHOD FOR PRODUCING LEUCINE USING THE SAME. Applicant: CJ CheilJedang Corporation. The sequence listing filed with the application follows.

SEQUENCE LISTING (14 sequences)

SEQ ID NO: 1 - protein, 367 aa, Corynebacterium glutamicum
MTSLEFTVTRTENPTSPDRLKEILAAPKFGKFFTDHMVTIDWNESEGWHNAQLVPYAPIPMDPATTVFHYGQAIFEGIKAYRHSDETIKTFRPDENAERMQRSAARMAMPQLPTEDFIKALELLVDADQDWVPEYGGEASLYLRPFMISTEIGLGVSPADAYKFLVIASPVGAYFTGGIKPVSVWLSEDYVRAAPGGTGDAKFAGNYAASLLAQSQAAEKGCDQVVWLDAIEHKYIEEMGGMNLGFIYRNGDQVKLVTPELSGSLLPGITRKSLLQVARDLGYEVEERKITTTEWEEDAKSGAMTEAFACGTAAVITPVGTVKSAHGTFEVNNNEVGEITMKLRETLTGIQQGNVEDQNGWLYPLVG

SEQ ID NO: 2 - DNA, 1104 bp, Corynebacterium glutamicum
atgacgtcattagagttcacagtaacccgtaccgaaaatccgacgtcacccgatcgtctgaaggaaattcttgccgcaccgaagttcggtaagttcttcaccgaccacatggtgaccattgactggaacgagtcggaaggctggcacaacgcccaattagtgccatacgcgccgattcctatggatcctgccaccaccgtattccactacggacaggcaatttttgagggaattaaggcctaccgccattcggacgaaaccatcaagactttccgtcctgatgaaaacgccgagcgtatgcagcgttcagcagctcgaatggcaatgccacagttgccaaccgaggactttattaaagcacttgaactgctggtagacgcggatcaggattgggttcctgagtacggcggagaagcttccctctacctgcgcccattcatgatctccaccgaaattggcttgggtgtcagcccagctgatgcctacaagttcctggtcatcgcatccccagtcggcgcttacttcaccggtggaatcaagcctgtttccgtctggctgagcgaagattacgtccgcgctgcacccggcggaactggtgacgccaaatttgctggcaactacgcggcttctttgcttgcccagtcccaggctgcggaaaagggctgtgaccaggtcgtatggttggatgccatcgagcacaagtacatcgaagaaatgggtggcatgaaccttgggttcatctaccgcaacggcgaccaagtcaagctagtcacccctgaactttccggctcactacttccaggcatcacccgcaagtcacttctacaagtagcacgcgacttgggatacgaagtagaagagcgaaagatcaccaccaccgagtgggaagaagacgcaaagtctggcgccatgaccgaggcatttgcttgcggtactgcagctgttatcacccctgttggcaccgtgaaatcagctcacggcaccttcgaagtgaacaacaatgaagtcggagaaatcacgatgaagcttcgtgaaaccctcaccggaattcagcaaggaaacgttgaagaccaaaacggatggctttacccactggttggctaa

SEQ ID NO: 3 - protein, 367 aa, Artificial Sequence
  Corynebacteirum glutamicum_ilvE_V156A
MTSLEFTVTRTENPTSPDRLKEILAAPKFGKFFTDHMVTIDWNESEGWHNAQLVPYAPIPMDPATTVFHYGQAIFEGIKAYRHSDETIKTFRPDENAERMQRSAARMAMPQLPTEDFIKALELLVDADQDWVPEYGGEASLYLRPFMISTEIGLGASPADAYKFLVIASPVGAYFTGGIKPVSVWLSEDYVRAAPGGTGDAKFAGNYAASLLAQSQAAEKGCDQVVWLDAIEHKYIEEMGGMNLGFIYRNGDQVKLVTPELSGSLLPGITRKSLLQVARDLGYEVEERKITTTEWEEDAKSGAMTEAFACGTAAVITPVGTVKSAHGTFEVNNNEVGEITMKLRETLTGIQQGNVEDQNGWLYPLVG

SEQ ID NO: 4 - DNA, 1104 bp, Artificial Sequence
  Corynebacteirum glutamicum_ilvE_V156A
atgacgtcattagagttcacagtaacccgtaccgaaaatccgacgtcacccgatcgtctgaaggaaattcttgccgcaccgaagttcggtaagttcttcaccgaccacatggtgaccattgactggaacgagtcggaaggctggcacaacgcccaattagtgccatacgcgccgattcctatggatcctgccaccaccgtattccactacggacaggcaatttttgagggaattaaggcctaccgccattcggacgaaaccatcaagactttccgtcctgatgaaaacgccgagcgtatgcagcgttcagcagctcgaatggcaatgccacagttgccaaccgaggactttattaaagcacttgaactgctggtagacgcggatcaggattgggttcctgagtacggcggagaagcttccctctacctgcgcccattcatgatctccaccgaaattggcttgggtgccagcccagctgatgcctacaagttcctggtcatcgcatccccagtcggcgcttacttcaccggtggaatcaagcctgtttccgtctggctgagcgaagattacgtccgcgctgcacccggcggaactggtgacgccaaatttgctggcaactacgcggcttctttgcttgcccagtcccaggctgcggaaaagggctgtgaccaggtcgtatggttggatgccatcgagcacaagtacatcgaagaaatgggtggcatgaaccttgggttcatctaccgcaacggcgaccaagtcaagctagtcacccctgaactttccggctcactacttccaggcatcacccgcaagtcacttctacaagtagcacgcgacttgggatacgaagtagaagagcgaaagatcaccaccaccgagtgggaagaagacgcaaagtctggcgccatgaccgaggcatttgcttgcggtactgcagctgttatcacccctgttggcaccgtgaaatcagctcacggcaccttcgaagtgaacaacaatgaagtcggagaaatcacgatgaagcttcgtgaaaccctcaccggaattcagcaaggaaacgttgaagaccaaaacggatggctttacccactggttggctaa

SEQ ID NO: 5 - DNA, 30 bp, Artificial Sequence
  primer
ctaatctcgaggtcacccgatcgtctgaag

SEQ ID NO: 6 - DNA, 27 bp, Artificial Sequence
  primer
gggtctagagtcttaaaaccggttgat

SEQ ID NO: 7 - DNA, 18 bp, Artificial Sequence
  primer
cgaggtcaactccaaggc

SEQ ID NO: 8 - DNA, 20 bp, Artificial Sequence
  primer
cgtaaagcttaaacgccgcc

SEQ ID NO: 9 - DNA, 19 bp, Artificial Sequence
  primer
gtcacccgatcgtctgaag

SEQ ID NO: 10 - DNA, 18 bp, Artificial Sequence
  primer
gtcttaaaaccggttgat

SEQ ID NO: 11 - DNA, 41 bp, Artificial Sequence
  primer
acccggggatcctctagagaatcttcgccttcaaaaatcgc

SEQ ID NO: 12 - DNA, 39 bp, Artificial Sequence
  primer
gtaggcatcagctgggctggcacccaagccaatttcggt

SEQ ID NO: 13 - DNA, 39 bp, Artificial Sequence
  primer
accgaaattggcttgggtgccagcccagctgatgcctac

SEQ ID NO: 14 - DNA, 42 bp, Artificial Sequence
  primer
aagcttgcatgcctgcagcttaaagtcacctacgttttgtac